European Patent Application EP 4 342 910 A1, published March 27, 2024. Title: Anti-Norovirus antibody. Applicant: DENKA COMPANY LIMITED. The sequence listing filed with the application follows.

SEQUENCE LISTING (4 sequences)

SEQ ID NO: 1 - protein, 23 aa, Artificial Sequence
  partial sequence of shell domain of Norovirus
MLYTPLRTGGGSGGTDPFVVAGR

SEQ ID NO: 2 - protein, 22 aa, Artificial Sequence
  partial sequence of shell domain of norovirus
PVAGASTAVATAGQVNMIDPWI

SEQ ID NO: 3 - protein, 23 aa, Artificial Sequence
  partial sequence of shell domain of norovirus
RLVAMLYTPLRANGSGDDVFTVS

SEQ ID NO: 4 - protein, 22 aa, Artificial Sequence
  partial sequence of shell domain of norovirus
AAPVTGQQNIIDPWIRNNFVQA